European Patent Application EP 4 141 021 A1, published March 1, 2023. Title: Antibacterial Protein CDL200 Having Lytic Activity to Clostridioides difficile. Applicant: iNtRON Biotechnology, Co. Ltd. The sequence listing filed with the application follows.

SEQUENCE LISTING (2 sequences)

SEQ ID NO: 1 - protein, 160 aa, Artificial Sequence
  Antibacterial protein CDL200
MVDIIKMLTKKKSYPNKNSPKFIVIHETDNEDKGADAKRHAQALNNGNLEASVHYYVDDKVIYQTLDHKDGAWAVGKSYGTALVAGVTNYNSINIEICVNRDGNYTKARQNAIDLTRKLMKDLNISTDKVIRHYDAKRKYCPRKMLDNPKLWVDFKDKIK

SEQ ID NO: 2 - DNA, 3711 bp, Artificial Sequence
  Gene coding Escherichia coli Top10-CDL200 to produce antibacterial protein CDL200
ccatcgaatggccagatgattaattcctaatttttgttgacactctatcattgatagagttattttaccactccctatcagtgatagagaaaagtgaaatgaatagttcgacaaaaatctagaaataattttgtttaactttaagaaggagatatacatatggttgatatcatcaagatgttaacgaaaaaaaagtcttacccaaataaaaattcgccgaagttcatcgtaattcacgaaaccgataacgaagataaaggtgcggatgcaaagcgccacgcgcaggccttgaataatgggaacttagaagcgtcagtccattactacgtagatgataaggttatctaccagacgttggaccataaagatggtgcatgggctgtgggcaaaagttacggaaccgcgcttgtggccggtgtcacgaattacaactccatcaacatagagatttgtgtaaatcgggacggaaattatacaaaggcgagacagaacgcaatcgaccttactcgtaagttgatgaaagacttgaacatatctactgataaagtcattcgccactatgatgcgaaacgcaaatactgcccccgtaagatgttagataaccccaaattgtgggtggatttcaaggacaagatcaagtagaattcgagctcggtacccggggatccctcgaggtcgacctgcagggggaccatggtctcagcgcttggagccacccgcagttcgaaaaataataagcttgacctgtgaagtgaaaaatggcgcacattgtgcgacattttttttgtctgccgtttaccgctactgcgtcacggatctccacgcgccctgtagcggcgcattaagcgcggcgggtgtggtggttacgcgcagcgtgaccgctacacttgccagcgccctagcgcccgctcctttcgctttcttcccttcctttctcgccacgttcgccggctttccccgtcaagctctaaatcgggggctccctttagggttccgatttagtgctttacggcacctcgaccccaaaaaacttgattagggtgatggttcacgtagtgggccatcgccctgatagacggtttttcgccctttgacgttggagtccacgttctttaatagtggactcttgttccaaactggaacaacactcaaccctatctcggtctattcttttgatttataagggattttgccgatttcggcctattggttaaaaaatgagctgatttaacaaaaatttaacgcgaattttaacaaaatattaacgcttacaatttcaggtggcacttttcggggaaatgtgcgcggaacccctatttgtttatttttctaaatacattcaaatatgtatccgctcatgagacaataaccctgataaatgcttcaataatattgaaaaaggaagagtatgagtattcaacatttccgtgtcgcccttattcccttttttgcggcattttgccttcctgtttttgctcacccagaaacgctggtgaaagtaaaagatgctgaagatcagttgggtgcacgagtgggttacatcgaactggatctcaacagcggtaagatccttgagagttttcgccccgaagaacgttttccaatgatgagcacttttaaagttctgctatgtggcgcggtattatcccgtattgacgccgggcaagagcaactcggtcgccgcatacactattctcagaatgacttggttgagtactcaccagtcacagaaaagcatcttacggatggcatgacagtaagagaattatgcagtgctgccataaccatgagtgataacactgcggccaacttacttctgacaacgatcggaggaccgaaggagctaaccgcttttttgcacaacatgggggatcatgtaactcgccttgatcgttgggaaccggagctgaatgaagccataccaaacgacgagcgtgacaccacgatgcctgtagcaatggcaacaacgttgcgcaaactattaactggcgaactacttactctagcttcccggcaacaattgatagactggatggaggcggataaagttgcaggaccacttctgcgctcggcccttccggctggctggtttattgctgataaatctggagccggtgagcgtggctctcgcggtatcattgcagcactggggccagatggtaagccctcccgtatcgtagttatctacacgacggggagtcaggcaactatggatgaacgaaatagacagatcgctgagataggtgcctcactgattaagcattggtaggaattaatgatgtctcgtttagataaaagtaaagtgattaacagcgcattagagctgcttaatgaggtcggaatcgaaggtttaacaacccgtaaactcgcccagaagctaggtgtagagcagcctacattgtattggcatgtaaaaaataagcgggctttgctcgacgccttagccattgagatgttagataggcaccatactcacttttgccctttagaaggggaaagctggcaagattttttacgtaataacgctaaaagttttagatgtgctttactaagtcatcgcgatggagcaaaagtacatttaggtacacggcctacagaaaaacagtatgaaactctcgaaaatcaattagcctttttatgccaacaaggtttttcactagagaatgcattatatgcactcagcgcagtggggcattttactttaggttgcgtattggaagatcaagagcatcaagtcgctaaagaagaaagggaaacacctactactgatagtatgccgccattattacgacaagctatcgaattatttgatcaccaaggtgcagagccagccttcttattcggccttgaattgatcatttgcggattagaaaaacaacttaaatgtgaaagtgggtcttaaaagcagcataacctttttccgtgatggtaacttcactagtttaaaaggatctaggtgaagatcctttttgataatctcatgaccaaaatcccttaacgtgagttttcgttccactgagcgtcagaccccgtagaaaagatcaaaggatcttcttgagatcctttttttctgcgcgtaatctgctgcttgcaaacaaaaaaaccaccgctaccagcggtggtttgtttgccggatcaagagctaccaactctttttccgaaggtaactggcttcagcagagcgcagataccaaatactgtccttctagtgtagccgtagttaggccaccacttcaagaactctgtagcaccgcctacatacctcgctctgctaatcctgttaccagtggctgctgccagtggcgataagtcgtgtcttaccgggttggactcaagacgatagttaccggataaggcgcagcggtcgggctgaacggggggttcgtgcacacagcccagcttggagcgaacgacctacaccgaactgagatacctacagcgtgagctatgagaaagcgccacgcttcccgaagggagaaaggcggacaggtatccggtaagcggcagggtcggaacaggagagcgcacgagggagcttccagggggaaacgcctggtatctttatagtcctgtcgggtttcgccacctctgacttgagcgtcgatttttgtgatgctcgtcaggggggcggagcctatggaaaaacgccagcaacgcggcctttttacggttcctggccttttgctggccttttgctcacatgacccgaca